European Patent Application EP 4 778 526 A1, published July 22, 2026. Title: Anti-aging agent, oral composition for anti-aging and use of compound. Applicant: INSTITUTE OF RHEOLOGICAL FUNCTION OF FOOD CO., LTD. Application JP. The sequence listing filed with the application follows.

SEQUENCE LISTING (18 sequences)

SEQ ID NO: 1 - DNA, 20 bp, synthetic construct
  source 1..20: mol_type = other DNA
gccagcagggaattttgtta

SEQ ID NO: 2 - DNA, 20 bp, synthetic construct
  source 1..20: mol_type = other DNA
tgtcaccttgccattcttga

SEQ ID NO: 3 - DNA, 20 bp, synthetic construct
  source 1..20: mol_type = other DNA
tcagtggctggaacagtgag

SEQ ID NO: 4 - DNA, 20 bp, synthetic construct
  source 1..20: mol_type = other DNA
agcgccatggaaaatgtaac

SEQ ID NO: 5 - DNA, 20 bp, synthetic construct
  source 1..20: mol_type = other DNA
gtccagatccctgtgagcat

SEQ ID NO: 6 - DNA, 20 bp, synthetic construct
  source 1..20: mol_type = other DNA
caatgtcaccacctccacag

SEQ ID NO: 7 - DNA, 20 bp, synthetic construct
  source 1..20: mol_type = other DNA
tgtctcgtgcagacttgacc

SEQ ID NO: 8 - DNA, 19 bp, synthetic construct
  source 1..19: mol_type = other DNA
tctgggcgaggtctaacag

SEQ ID NO: 9 - DNA, 20 bp, synthetic construct
  source 1..20: mol_type = other DNA
attggttccaagacgcgtag

SEQ ID NO: 10 - DNA, 20 bp, synthetic construct
  source 1..20: mol_type = other DNA
attggcaccaagctatccac

SEQ ID NO: 11 - DNA, 21 bp, synthetic construct
  source 1..21: mol_type = other DNA
agtccctgccctttgtacaca

SEQ ID NO: 12 - DNA, 19 bp, synthetic construct
  source 1..19: mol_type = other DNA
cgatccgagggcctcacta

SEQ ID NO: 13 - DNA, 20 bp, synthetic construct
  source 1..20: mol_type = other DNA
cataggggcatctgctcatt

SEQ ID NO: 14 - DNA, 20 bp, synthetic construct
  source 1..20: mol_type = other DNA
gctgctggaacagaatagcc

SEQ ID NO: 15 - DNA, 20 bp, synthetic construct
  source 1..20: mol_type = other DNA
agttccagccgtctctgtgt

SEQ ID NO: 16 - DNA, 20 bp, synthetic construct
  source 1..20: mol_type = other DNA
gatcctttggattcctgcaa

SEQ ID NO: 17 - DNA, 20 bp, synthetic construct
  source 1..20: mol_type = other DNA
gatctggcaccacaccttct

SEQ ID NO: 18 - DNA, 20 bp, synthetic construct
  source 1..20: mol_type = other DNA
ggggtgttgaaggtctcaaa